European Patent Specification EP 4 158 356 B1, published April 10, 2024. Title: IN VITRO METHOD AND KIT FOR THE PROGNOSIS OF AMYOTROPHIC LATERAL SCLEROSIS. Applicant: Universidad del Pais Vasco/Euskal Herriko Unibersitatea Administración General de la Comunidad Autónoma de Euskadi Fundació Institut de Recerca Biomédica de Bellvitge (IDIBELL). The sequence listing filed with the application follows.

SEQUENCE LISTING (3 sequences)

SEQ ID NO: 1 - DNA, 21 bp, Artificial sequence
  Artificial sequence
ccagttaagaattgtatttaa

SEQ ID NO: 2 - DNA, 21 bp, Artificial sequence
  Artificial sequence
ctggacatgggtgttctacta

SEQ ID NO: 3 - DNA, 392 bp, Artificial sequence
  Artificial sequence
ctccgcagatccagcattataagtgcacaatctttataactaaactttcttagcgtaagccaaaatatatttaataaacaacaaaatacaaatcaaattctacttaagtgatacaatgatacaatttttactgagctttggcgcagaatttattttgaagtgtgttttatcaattgtgttattagccatccagtgtcatcttgtttacaattatcaaaatatctattacatattaaatacaattcttaactggtttgtatgtggaatacatatatgtaaatttaagtaagctacagaggtgttggttaaccacattaaccacatcattgggtgacaggcaccgccttaaagaaagtttgacttctccgcggcgttttgagatccgctgctct